European Patent Application EP 4 596 691 A1, published August 6, 2025. Title: Random sgRNA Library Generation Using Total mRNA via Enzymatic Reactions. Applicant: POSTECH Research and Business Development Foundation. The sequence listing filed with the application follows.

SEQUENCE LISTING (132 sequences)

SEQ ID NO: 1 - DNA, 30 bp, synthetic construct
  source 1..30: mol_type = other DNA
  misc_feature 17..22: note = EcoP15I restriction emzyme recognition site
aggtatctcgagtccccagcagcnnnnnnn

SEQ ID NO: 2 - DNA, 30 bp, synthetic construct
  source 1..30: mol_type = other DNA
  misc_feature 20..23: note = SfiI restriction enzyme partial recognition site
  misc_feature 29..30: note = SfiI restriction enzyme partial recognition site
  misc_feature 28..30: note = RNA
  misc_feature 1..27: note = DNA
agtggtatcaacgcagagtggccaagcggg

SEQ ID NO: 3 - DNA, 30 bp, synthetic construct; identical to SEQ ID NO: 2
  source 1..30: mol_type = other DNA
  misc_feature 1..27: note = DNA
  misc_feature 28..30: note = RNA
  misc_feature 29..30: note = BamHI restriction enzyme partial recognition site

SEQ ID NO: 4 - DNA, 30 bp, synthetic construct; identical to SEQ ID NO: 2
  source 1..30: mol_type = other DNA
  misc_feature 1..27: note = DNA
  misc_feature 28..30: note = RNA
  misc_feature 30: note = KpnI restriction enzyme partial recognition site

SEQ ID NO: 5 - DNA, 30 bp, synthetic construct
  source 1..30: mol_type = other DNA
  misc_binding 1: bound_moiety = Biotin
  misc_feature 17..22: note = AcuI restriction enzyme recognition site
  misc_feature 24..29: note = EcoP15I restriction enzyme recognition site
aggctcactgcatatgctgaagtcagcagc

SEQ ID NO: 6 - DNA, 28 bp, synthetic construct
  source 1..28: mol_type = other DNA
  misc_binding 1: bound_moiety = Biotin
  misc_feature 15..20: note = AcuI restriction enzyme recognition site
  misc_feature 24..28: note = EcoP15I restriction enzyme partial recognition site
aggctcactgcatactgaagtgtcagca

SEQ ID NO: 7 - DNA, 33 bp, synthetic construct
  source 1..33: mol_type = other DNA
  misc_binding 1: bound_moiety = Biotin
  misc_feature 17..22: note = AcuI restriction enzyme recognition site
  misc_feature 24..29: note = EcoP15I restriction enzyme recognition site
aggctcactgcatatgctgaagtcagcaggtac

SEQ ID NO: 8 - DNA, 27 bp, synthetic construct
  source 1..27: mol_type = other DNA
gctgacttcagcatatgcagtgagcct

SEQ ID NO: 9 - DNA, 32 bp, synthetic construct
  source 1..32: mol_type = other DNA
gatctgctgacacttcagtatgcagtgagcct

SEQ ID NO: 10 - DNA, 28 bp, synthetic construct
  source 1..28: mol_type = other DNA
tgctgacttcagcatatgcagtgagcct

SEQ ID NO: 11 - DNA, 40 bp, synthetic construct
  source 1..40: mol_type = other DNA
gatctttgacagctagctcagtcctaggtataatactagt

SEQ ID NO: 12 - DNA, 42 bp, synthetic construct
  source 1..42: mol_type = other DNA
nnactagtattatacctaggactgagctagctgtcaaagatc

SEQ ID NO: 13 - DNA, 40 bp, synthetic construct
  source 1..40: mol_type = other DNA
gttttagagctagaaatagcaagttaaaataaggctagtc

SEQ ID NO: 14 - DNA, 42 bp, synthetic construct
  source 1..42: mol_type = other DNA
gactagccttattttaacttgctatttctagctctaaaacnn

SEQ ID NO: 15 - DNA, 32 bp, synthetic construct
  source 1..32: mol_type = other DNA
cttcttcctgttaccgttcgacttgcatgtgt

SEQ ID NO: 16 - DNA, 32 bp, synthetic construct
  source 1..32: mol_type = other DNA
gcctgccgccagcgttcaatctgagccatgat

SEQ ID NO: 17 - DNA, 32 bp, synthetic construct
  source 1..32: mol_type = other DNA
cgtttccagtagttatccccctccatcaggca

SEQ ID NO: 18 - DNA, 32 bp, synthetic construct
  source 1..32: mol_type = other DNA
acattactcacccgtccgccactcgtcagcaa

SEQ ID NO: 19 - DNA, 32 bp, synthetic construct
  source 1..32: mol_type = other DNA
taatcccatctgggcacatccgatggcaagag

SEQ ID NO: 20 - DNA, 32 bp, synthetic construct
  source 1..32: mol_type = other DNA
tccccctctttggtcttgcgacgttatgcggt

SEQ ID NO: 21 - DNA, 32 bp, synthetic construct
  source 1..32: mol_type = other DNA
gtctcagttccagtgtggctggtcatcctctc

SEQ ID NO: 22 - DNA, 32 bp, synthetic construct
  source 1..32: mol_type = other DNA
agggatcgtcgcctaggtgagccgttacccca

SEQ ID NO: 23 - DNA, 32 bp, synthetic construct
  source 1..32: mol_type = other DNA
catacacgcggcatggctgcatcaggcttgcg

SEQ ID NO: 24 - DNA, 32 bp, synthetic construct
  source 1..32: mol_type = other DNA
caatattccccactgctgcctcccgtaggagt

SEQ ID NO: 25 - DNA, 32 bp, synthetic construct
  source 1..32: mol_type = other DNA
gcgggtaacgtcaatgagcaaaggtattaact

SEQ ID NO: 26 - DNA, 32 bp, synthetic construct
  source 1..32: mol_type = other DNA
tcctccccgctgaaagtactttacaacccgaa

SEQ ID NO: 27 - DNA, 32 bp, synthetic construct
  source 1..32: mol_type = other DNA
tttacgcccagtaattccgattaacgcttgca

SEQ ID NO: 28 - DNA, 32 bp, synthetic construct
  source 1..32: mol_type = other DNA
ttaccgcggctgctggcacggagttagccggt

SEQ ID NO: 29 - DNA, 32 bp, synthetic construct
  source 1..32: mol_type = other DNA
ctcaagcttgccagtatcagatgcagttccca

SEQ ID NO: 30 - DNA, 32 bp, synthetic construct
  source 1..32: mol_type = other DNA
cggggatttcacatctgacttaacaaaccgcc

SEQ ID NO: 31 - DNA, 32 bp, synthetic construct
  source 1..32: mol_type = other DNA
ggggccgccttcgccaccggtattcctccaga

SEQ ID NO: 32 - DNA, 32 bp, synthetic construct
  source 1..32: mol_type = other DNA
atttcaccgctacacctggaattctacccccc

SEQ ID NO: 33 - DNA, 32 bp, synthetic construct
  source 1..32: mol_type = other DNA
atcgtttacggcgtggactaccagggtatcta

SEQ ID NO: 34 - DNA, 32 bp, synthetic construct
  source 1..32: mol_type = other DNA
gctccccacgctttcgcacctgagcgtcagtc

SEQ ID NO: 35 - DNA, 32 bp, synthetic construct
  source 1..32: mol_type = other DNA
cttgcggccgtactccccaggcggtcgactta

SEQ ID NO: 36 - DNA, 32 bp, synthetic construct
  source 1..32: mol_type = other DNA
ctccggaagccacgcctcaagggcacaacctc

SEQ ID NO: 37 - DNA, 32 bp, synthetic construct
  source 1..32: mol_type = other DNA
gtaaggttcttcgcgttgcatcgaattaaacc

SEQ ID NO: 38 - DNA, 32 bp, synthetic construct
  source 1..32: mol_type = other DNA
accgcttgtgcgggcccccgtcaattcatttg

SEQ ID NO: 39 - DNA, 32 bp, synthetic construct
  source 1..32: mol_type = other DNA
gacgacagccatgcagcacctgtctcacggtt

SEQ ID NO: 40 - DNA, 32 bp, synthetic construct
  source 1..32: mol_type = other DNA
acattctcatctctgaaaacttccgtggatgt

SEQ ID NO: 41 - DNA, 32 bp, synthetic construct
  source 1..32: mol_type = other DNA
agttcccggccggaccgctggcaacaaaggat

SEQ ID NO: 42 - DNA, 32 bp, synthetic construct
  source 1..32: mol_type = other DNA
gctcgttgcgggacttaacccaacatttcaca

SEQ ID NO: 43 - DNA, 32 bp, synthetic construct
  source 1..32: mol_type = other DNA
gtgtgtagccctggtcgtaagggccatgatga

SEQ ID NO: 44 - DNA, 32 bp, synthetic construct
  source 1..32: mol_type = other DNA
atccccaccttcctccagtttatcactggcag

SEQ ID NO: 45 - DNA, 32 bp, synthetic construct
  source 1..32: mol_type = other DNA
ctccaatccggactacgacgcactttatgagg

SEQ ID NO: 46 - DNA, 32 bp, synthetic construct
  source 1..32: mol_type = other DNA
tctcgcgaggtcgcttctctttgtatgcgcca

SEQ ID NO: 47 - DNA, 32 bp, synthetic construct
  source 1..32: mol_type = other DNA
tacaaggcccgggaacgtattcaccgtggcat

SEQ ID NO: 48 - DNA, 32 bp, synthetic construct
  source 1..32: mol_type = other DNA
cgattactagcgattccgacttcatggagtcg

SEQ ID NO: 49 - DNA, 32 bp, synthetic construct
  source 1..32: mol_type = other DNA
tcacaaagtggtaagcgccctcccgaaggtta

SEQ ID NO: 50 - DNA, 32 bp, synthetic construct
  source 1..32: mol_type = other DNA
cttcttttgcaacccactcccatggtgtgacg

SEQ ID NO: 51 - DNA, 32 bp, synthetic construct
  source 1..32: mol_type = other DNA
ccgcaggttcccctacggttaccttgttacga

SEQ ID NO: 52 - DNA, 32 bp, synthetic construct
  source 1..32: mol_type = other DNA
accgacgcttatcgcagattagcacgtccttc

SEQ ID NO: 53 - DNA, 32 bp, synthetic construct
  source 1..32: mol_type = other DNA
gactgccagggcatccaccgtgtacgcttagt

SEQ ID NO: 54 - DNA, 32 bp, synthetic construct
  source 1..32: mol_type = other DNA
ggattcagttaatgatagtgtgtcgaaacaca

SEQ ID NO: 55 - DNA, 32 bp, synthetic construct
  source 1..32: mol_type = other DNA
cccattcggaaatcgccggttataacggttca

SEQ ID NO: 56 - DNA, 32 bp, synthetic construct
  source 1..32: mol_type = other DNA
gctactgggggaatctcggttgatttcttttc

SEQ ID NO: 57 - DNA, 32 bp, synthetic construct
  source 1..32: mol_type = other DNA
cttagatgtttcagttcccccggttcgcctca

SEQ ID NO: 58 - DNA, 32 bp, synthetic construct
  source 1..32: mol_type = other DNA
accctgtatcgcgcgcctttccagacgcttcc

SEQ ID NO: 59 - DNA, 32 bp, synthetic construct
  source 1..32: mol_type = other DNA
cacactgattcaggctctgggctgctccccgt

SEQ ID NO: 60 - DNA, 32 bp, synthetic construct
  source 1..32: mol_type = other DNA
cccccatattcagacaggataccacgtgtccc

SEQ ID NO: 61 - DNA, 32 bp, synthetic construct
  source 1..32: mol_type = other DNA
atcgagctcacagcatgtgcatttttgtgtac

SEQ ID NO: 62 - DNA, 32 bp, synthetic construct
  source 1..32: mol_type = other DNA
tcgccggggttcttttcgcctttccctcacgg

SEQ ID NO: 63 - DNA, 32 bp, synthetic construct
  source 1..32: mol_type = other DNA
actatcggtcagtcaggagtatttagccttgg

SEQ ID NO: 64 - DNA, 32 bp, synthetic construct
  source 1..32: mol_type = other DNA
tatacaaaaggtacgcagtcacacgcctaagc

SEQ ID NO: 65 - DNA, 32 bp, synthetic construct
  source 1..32: mol_type = other DNA
ctgcttgtacgtacacggtttcaggttctttt

SEQ ID NO: 66 - DNA, 32 bp, synthetic construct
  source 1..32: mol_type = other DNA
cttaacgcccagttaagactcggtttcccttc

SEQ ID NO: 67 - DNA, 32 bp, synthetic construct
  source 1..32: mol_type = other DNA
attcggttaaccttgctacagaatataagtcg

SEQ ID NO: 68 - DNA, 32 bp, synthetic construct
  source 1..32: mol_type = other DNA
cggttcggtcctccagttagtgttacccaacc

SEQ ID NO: 69 - DNA, 32 bp, synthetic construct
  source 1..32: mol_type = other DNA
cccatggctagatcaccgggtttcgggtctat

SEQ ID NO: 70 - DNA, 32 bp, synthetic construct
  source 1..32: mol_type = other DNA
ttcggggagaaccagctatctcccggtttgat

SEQ ID NO: 71 - DNA, 32 bp, synthetic construct
  source 1..32: mol_type = other DNA
acccccagccacaagtcatccgctaatttttc

SEQ ID NO: 72 - DNA, 32 bp, synthetic construct
  source 1..32: mol_type = other DNA
ggttggtaagtcgggatgacccccttgccgaa

SEQ ID NO: 73 - DNA, 32 bp, synthetic construct
  source 1..32: mol_type = other DNA
tacccccggagatgaattcacgaggcgctacc

SEQ ID NO: 74 - DNA, 32 bp, synthetic construct
  source 1..32: mol_type = other DNA
ttgtttccctcttcacgacggacgttagcacc

SEQ ID NO: 75 - DNA, 32 bp, synthetic construct
  source 1..32: mol_type = other DNA
tctcccgtgataacattctccggtattcgcag

SEQ ID NO: 76 - DNA, 32 bp, synthetic construct
  source 1..32: mol_type = other DNA
taagccaacatcctggctgtctgggccttccc

SEQ ID NO: 77 - DNA, 32 bp, synthetic construct
  source 1..32: mol_type = other DNA
ccacttaaccatgactttgggaccttagctgg

SEQ ID NO: 78 - DNA, 32 bp, synthetic construct
  source 1..32: mol_type = other DNA
catggtttagccccgttacatcttccgcgcag

SEQ ID NO: 79 - DNA, 32 bp, synthetic construct
  source 1..32: mol_type = other DNA
ccagtgagctattacgctttctttaaatgatg

SEQ ID NO: 80 - DNA, 32 bp, synthetic construct
  source 1..32: mol_type = other DNA
atgcctcacagcacaccttcgcaggcttacag

SEQ ID NO: 81 - DNA, 32 bp, synthetic construct
  source 1..32: mol_type = other DNA
tacccaacaacgcataagcgtcgctgccgcag

SEQ ID NO: 82 - DNA, 32 bp, synthetic construct
  source 1..32: mol_type = other DNA
aacccttggtcttccggcgagcgggcttttca

SEQ ID NO: 83 - DNA, 32 bp, synthetic construct
  source 1..32: mol_type = other DNA
cgttacttatgtcagcattcgcacttctgata

SEQ ID NO: 84 - DNA, 32 bp, synthetic construct
  source 1..32: mol_type = other DNA
tattaacctgtttcccatcgactacgcctttc

SEQ ID NO: 85 - DNA, 32 bp, synthetic construct
  source 1..32: mol_type = other DNA
taggggtcgactcaccctgccccgattaacgt

SEQ ID NO: 86 - DNA, 32 bp, synthetic construct
  source 1..32: mol_type = other DNA
tacacgcttaaaccgggacaaccgtcgcccgg

SEQ ID NO: 87 - DNA, 32 bp, synthetic construct
  source 1..32: mol_type = other DNA
cttctccgtccccccttcgcagtaacaccaag

SEQ ID NO: 88 - DNA, 32 bp, synthetic construct
  source 1..32: mol_type = other DNA
agggcatttgttgcttcagcaccgtagtgcct

SEQ ID NO: 89 - DNA, 32 bp, synthetic construct
  source 1..32: mol_type = other DNA
cctcagccttgattttccggatttgcctggaa

SEQ ID NO: 90 - DNA, 32 bp, synthetic construct
  source 1..32: mol_type = other DNA
ttggtattctctacctgaccacctgtgtcggt

SEQ ID NO: 91 - DNA, 32 bp, synthetic construct
  source 1..32: mol_type = other DNA
atttgatgttacctgatgcttagaggcttttc

SEQ ID NO: 92 - DNA, 32 bp, synthetic construct
  source 1..32: mol_type = other DNA
ctcacctacatatcagcgtgccttctcccgaa

SEQ ID NO: 93 - DNA, 32 bp, synthetic construct
  source 1..32: mol_type = other DNA
cattttgcctagttccttcacccgagttctct

SEQ ID NO: 94 - DNA, 32 bp, synthetic construct
  source 1..32: mol_type = other DNA
gtgtttgcacagtgctgtgtttttaataaaca

SEQ ID NO: 95 - DNA, 32 bp, synthetic construct
  source 1..32: mol_type = other DNA
ctggtatcttcgactgatttcagctccatccg

SEQ ID NO: 96 - DNA, 32 bp, synthetic construct
  source 1..32: mol_type = other DNA
cgatcaagagcttcgcttgcgctaaccccatc

SEQ ID NO: 97 - DNA, 32 bp, synthetic construct
  source 1..32: mol_type = other DNA
cggcaccgggcaggcgtcacaccgtatacgtc

SEQ ID NO: 98 - DNA, 32 bp, synthetic construct
  source 1..32: mol_type = other DNA
ttcgtgcaggtcggaacttacccgacaaggaa

SEQ ID NO: 99 - DNA, 32 bp, synthetic construct
  source 1..32: mol_type = other DNA
taggaccgttatagttacggccgccgtttacc

SEQ ID NO: 100 - DNA, 32 bp, synthetic construct
  source 1..32: mol_type = other DNA
ttgccgcgggtacactgcatcttcacagcgag

SEQ ID NO: 101 - DNA, 32 bp, synthetic construct
  source 1..32: mol_type = other DNA
tgagtctcgggtggagacagcctggccatcat

SEQ ID NO: 102 - DNA, 32 bp, synthetic construct
  source 1..32: mol_type = other DNA
tcaaagcctcccacctatcctacacatcaagg

SEQ ID NO: 103 - DNA, 32 bp, synthetic construct
  source 1..32: mol_type = other DNA
gtgtcaagctatagtaaaggttcacggggtct

SEQ ID NO: 104 - DNA, 32 bp, synthetic construct
  source 1..32: mol_type = other DNA
cggattacgggtcaacgttagaacatcaaaca

SEQ ID NO: 105 - DNA, 32 bp, synthetic construct
  source 1..32: mol_type = other DNA
tatttcaaggtcggctccatgcagactggcgt

SEQ ID NO: 106 - DNA, 32 bp, synthetic construct
  source 1..32: mol_type = other DNA
ttagccaaccttcgtgctcctccgttactctt

SEQ ID NO: 107 - DNA, 32 bp, synthetic construct
  source 1..32: mol_type = other DNA
cgccccagtcaaactacccaccagacactgtc

SEQ ID NO: 108 - DNA, 32 bp, synthetic construct
  source 1..32: mol_type = other DNA
gctttcgcacctgctcgcgccgtcacgctcgc

SEQ ID NO: 109 - DNA, 32 bp, synthetic construct
  source 1..32: mol_type = other DNA
cttatgccattgcactaacctcctgatgtccg

SEQ ID NO: 110 - DNA, 32 bp, synthetic construct
  source 1..32: mol_type = other DNA
gtatcagcctgttatccccggagtacctttta

SEQ ID NO: 111 - DNA, 32 bp, synthetic construct
  source 1..32: mol_type = other DNA
atggcccttccattcagaaccaccggatcact

SEQ ID NO: 112 - DNA, 32 bp, synthetic construct
  source 1..32: mol_type = other DNA
ccttgggacctacttcagccccaggatgtgat

SEQ ID NO: 113 - DNA, 32 bp, synthetic construct
  source 1..32: mol_type = other DNA
gaggtgccaaacaccgccgtcgatatgaactc

SEQ ID NO: 114 - DNA, 32 bp, synthetic construct
  source 1..32: mol_type = other DNA
gcccacggcagatagggaccgaactgtctcac

SEQ ID NO: 115 - DNA, 32 bp, synthetic construct
  source 1..32: mol_type = other DNA
cccagctcgcgtaccactttaaatggcgaaca

SEQ ID NO: 116 - DNA, 32 bp, synthetic construct
  source 1..32: mol_type = other DNA
cattggcatgacaacccgaacaccagtgatgc

SEQ ID NO: 117 - DNA, 32 bp, synthetic construct
  source 1..32: mol_type = other DNA
tcctctcgtactaggagcagcccccctcagtt

SEQ ID NO: 118 - DNA, 32 bp, synthetic construct
  source 1..32: mol_type = other DNA
agggagaactcatctcggggcaagtttcgtgc

SEQ ID NO: 119 - DNA, 32 bp, synthetic construct
  source 1..32: mol_type = other DNA
cagcacttatctcttccgcatttagctaccgg

SEQ ID NO: 120 - DNA, 32 bp, synthetic construct
  source 1..32: mol_type = other DNA
tagctcaacgcatcgctgcgcttacacacccg

SEQ ID NO: 121 - DNA, 32 bp, synthetic construct
  source 1..32: mol_type = other DNA
tcgtcgtcttcaacgttccttcaggaccctta

SEQ ID NO: 122 - DNA, 32 bp, synthetic construct
  source 1..32: mol_type = other DNA
aaggttaagcctcacggttcattagtaccggt

SEQ ID NO: 123 - DNA, 32 bp, synthetic construct
  source 1..32: mol_type = other DNA
cggcatggggtcaggtgggaccaccgcgctac

SEQ ID NO: 124 - DNA, 33 bp, synthetic construct
  source 1..33: mol_type = other DNA
cacactaccatcggcgctacggcgtttcacttc

SEQ ID NO: 125 - DNA, 32 bp, synthetic construct
  source 1..32: mol_type = other DNA
atgcctggcagttccctactctcgcatgggga

SEQ ID NO: 126 - DNA, 23 bp, synthetic construct
  source 1..23: mol_type = other DNA
agtggtatcaacgcagagtggcc

SEQ ID NO: 127 - DNA, 23 bp, synthetic construct
  source 1..23: mol_type = other DNA
aggtatctcgagtccccagcagc

SEQ ID NO: 128 - DNA, 31 bp, synthetic construct
  source 1..31: mol_type = other DNA
aggctcactgcatatgctgaagtcagcagcg

SEQ ID NO: 129 - DNA, 28 bp, synthetic construct
  source 1..28: mol_type = other DNA
gatctttgacagctagctcagtcctagg

SEQ ID NO: 130 - DNA, 34 bp, synthetic construct
  source 1..34: mol_type = other DNA
gactagccttattttaacttgctatttctagctc

SEQ ID NO: 131 - DNA, 35 bp, synthetic construct
  source 1..35: mol_type = other DNA
gttttagagctagaaatagcaagttaaaataaggc

SEQ ID NO: 132 - DNA, 31 bp, synthetic construct
  source 1..31: mol_type = other DNA
actagtattatacctaggactgagctagctg